European Patent Application EP 4 483 900 A1, published January 1, 2025. Title: Anticancer agent and screening method for anticancer agent. Applicant: INSTITUTE OF RHEOLOGICAL FUNCTION OF FOOD CO., LTD. Application WO. The sequence listing filed with the application follows.

SEQUENCE LISTING (1 sequence)

SEQ ID NO: 1 - RNA, 19 nt, synthetic construct
  misc_feature 1..19: note = siRNA for ATP8B2
  source 1..19: mol_type = other RNA
ggtgcttcgggctggtcat